European Patent Application EP 4 752 155 A1, published June 3, 2026. Title: CELLULAR IRON BIOSENSORS. Applicant: Medizinische Universität Graz. Application EP. The sequence listing filed with the application follows.

SEQUENCE LISTING (32 sequences)

SEQ ID NO: 1 - DNA, 505 bp, synthetic construct
  source 1..505: mol_type = other DNA
gggttgcgccttttccaaggcagccctgggtttgcgcagggacgcggctgctctgggcgtggttccgggaaacgcagcggcgccgaccctgggtctcgcacattcttcacgtccgttcgcagcgtcacccggatcttcgccgctacccttgtgggccccccggcgacgcttcctgctccgcccctaagtcgggaaggttccttgcggttcgcggcgtgccggacgtgacaaacggaagccgcacgtctcactagtaccctcgcagacggacagcgccagggagcaatggcagcgcgccgaccgcgatgggctgtggccaatagcggctgctcagcagggcgcgccgagagcagcggccgggaaggggcggtgcgggaggcggggtgtggggcggtagtgtgggccctgttcctgcccgcgcggtgttccgcattctgcaagcctccggagcgcacgtcggcagtcggctccctcgttgaccgaatcaccgacctctctccccagg

SEQ ID NO: 2 - protein, 9 aa, synthetic construct
  VARIANT 1: note = X = any amino acid or absent
  VARIANT 5: note = X = any amino acid or absent
XDVEXNPGP

SEQ ID NO: 3 - protein, 25 aa, synthetic construct
  VARIANT 4: note = X = any amino acid or absent
  VARIANT 5: note = X = any amino acid or absent
  VARIANT 6: note = X = any amino acid or absent
  VARIANT 7: note = X = any amino acid or absent
  VARIANT 8: note = X = any amino acid or absent
  VARIANT 9: note = X = any amino acid or absent
  VARIANT 10: note = X = any amino acid or absent
  VARIANT 11: note = X = any amino acid or absent
  VARIANT 14: note = X = any amino acid or absent
  VARIANT 15: note = X = any amino acid or absent
  VARIANT 16: note = X = any amino acid or absent
  VARIANT 17: note = X = any amino acid or absent
  VARIANT 21: note = X = any amino acid or absent
GSGXXXXXXXXLLXXXXDVEXNPGP

SEQ ID NO: 4 - protein, 21 aa, synthetic construct
GSGEGRGSLLTCGDVEENPGP

SEQ ID NO: 5 - DNA, 63 bp, synthetic construct
  source 1..63: mol_type = other DNA
ggaagcggagagggcaggggaagtcttctaacatgcggggacgtggaggaaaatcccggcccc

SEQ ID NO: 6 - protein, 10 aa, synthetic construct
TIYNVHSDNK

SEQ ID NO: 7 - DNA, 30 bp, synthetic construct
  source 1..30: mol_type = other DNA
accatttataatgtacattctgacaataaa

SEQ ID NO: 8 - protein, 160 aa, synthetic construct
MAPFPEEVDVFTAPHWRMKQLVGLYCDKLSKTNFSNNNDFRALLQSLYATFKEFKMHEQIENEYIIGLLQQRSQTIYNVHSDNKLSEMLSLFEKGLKNVKNEYEQLNYAKQLKERLEAFTRDFLPHMKEEEEVFQPMLMEYFTYEELKDIKKKVIAQHCS

SEQ ID NO: 9 - DNA, 480 bp, synthetic construct
  source 1..480: mol_type = other DNA
atggcgccctttcctgaagaagtggacgtcttcaccgccccacactggcggatgaagcagctggtggggctctactgcgacaagctttctaaaaccaatttttccaacaacaacgatttccgtgctcttctgcagtctttgtatgctactttcaaggagttcaaaatgcatgagcagattgaaaatgaatacattattggtttgcttcaacaacgcagccagaccatttataatgtacattctgacaataaactctccgagatgcttagcctctttgaaaagggactgaagaatgttaagaatgaatatgaacagttaaattatgcaaaacaactgaaagagagattggaggcttttacaagagattttcttcctcacatgaaagaggaagaggaggtttttcagcccatgttaatggaatattttacctatgaagagcttaaggatattaaaaagaaagtgattgcacaacactgctct

SEQ ID NO: 10 - protein, 237 aa, synthetic construct
MVSKGEELIKENMHMKLYMEGTVDNHHFKCTSEGEGKPYEGTQTMRIKVVEGGPLPFAFDILATSFLYGSKTFINHTQGIPDFFKQSFPEGFTWERVTTYEDGGVLTATQDTSLQDGCLIYNVKIRGVNFTSNGPVMQKKTLGWEAFTETLYPADGGLEGRNDMALKLVGGSHLIANAKTTYRSKKPAKNLKMPGVYYVDYRLERIKEANNETYVEQHEVAVARYCDLPSKLGHKLN

SEQ ID NO: 11 - DNA, 714 bp, synthetic construct
  source 1..714: mol_type = other DNA
atggtgtctaagggcgaagagctgattaaggagaacatgcacatgaagctgtacatggagggcaccgtggacaaccatcacttcaagtgcacatccgagggcgaaggcaagccctacgagggcacccagaccatgagaatcaaggtggtcgagggcggccctctccccttcgccttcgacatcctggctactagcttcctctacggcagcaagaccttcatcaaccacacccagggcatccccgacttcttcaagcagtccttccctgagggcttcacatgggagagagtcaccacatacgaagacgggggcgtgctgaccgctacccaggacaccagcctccaggacggctgcctcatctacaacgtcaagatcagaggggtgaacttcacatccaacggccctgtgatgcagaagaaaacactcggctgggaggccttcaccgagacgctgtaccccgctgacggcggcctggaaggcagaaacgacatggccctgaagctcgtgggcgggagccatctgatcgcaaacgccaagaccacatatagatccaagaaacccgctaagaacctcaagatgcctggcgtctactatgtggactacagactggaaagaatcaaggaggccaacaacgagacctacgtcgagcagcacgaggtggcagtggccagatactgcgacctccctagcaaactggggcacaagcttaattaa

SEQ ID NO: 12 - protein, 236 aa, synthetic construct
MVSKGEEDNMASLPATHELHIFGSINGVDFDMVGQGTGNPNDGYEELNLKSTKGDLQFSPWILVPHIGYGFHQYLPYPDGMSPFQAAMVDGSGYQVHRTMQFEDGASLTVNYRYTYEGSHIKGEAQVKGTGFPADGPVMTNSLTAADWCRSKKTYPNDKTIISTFKWSYTTGNGKRYRSTARTTYTFAKPMAANYLKNQPMYVFRKTELKHSKTELNFKEWQKAFTDVMGMDELYK

SEQ ID NO: 13 - DNA, 708 bp, synthetic construct
  source 1..708: mol_type = other DNA
atggtgagtaagggggaggaagataacatggcctcacttccagcgactcacgaacttcacatttttgggtccatcaatggcgtggatttcgatatggtagggcaagggactggcaaccctaacgacggttacgaagaactcaatctgaaatcaacgaaaggggatttgcaattttccccatggatactcgtcccccatataggctatggattccaccaatatctgccgtatccagacggaatgtctccgtttcaagccgcaatggtagacggtagcggttaccaggtccaccggacgatgcaattcgaagatggggcctccctgacagtaaattatagatatacctatgaagggagtcacataaagggagaagctcaggtcaaaggaacgggtttcccggctgacggaccggtgatgaccaattcactgaccgccgccgattggtgccgctctaaaaaaacttacccaaatgataagactatcatttcaacttttaaatggagttacactacggggaatggtaagaggtacaggtcaacagccaggacaacttacacatttgccaagccaatggcggcgaactatttgaaaaatcagccaatgtacgttttccgaaaaaccgaattgaaacattctaagaccgagcttaatttcaaggaatggcaaaaagcatttacggatgtgatggggatggatgagctttacaag

SEQ ID NO: 14 - protein, 236 aa, synthetic construct
MVSKGEEDNMAIIKEFMRFKVHMEGSVNGHEFEIEGEGEGRPYEGTQTAKLKVTKGGPLPFAWDILSPQFMYGSKAYVKHPADIPDYLKLSFPEGFKWERVMNFEDGGVVTVTQDSSLQDGEFIYKVKLRGTNFPSDGPVMQKKTMGWEASSERMYPEDGALKGEIKQRLKLKDGGHYDAEVKTTYKAKKPVQLPGAYNVNIKLDITSHNEDYTIVEQYERAEGRHSTGGMDELYK

SEQ ID NO: 15 - DNA, 714 bp, synthetic construct
  source 1..714: mol_type = other DNA
atggtctccaaaggagaggaagacaatatggccattatcaaagagtttatgcgatttaaagtgcacatggagggaagcgtcaacgggcatgagtttgagattgagggggaaggagagggaagaccttatgaagggacccagactgccaaactgaaagtcaccaagggcggacccctgccatttgcttgggacattctgagcccacaattcatgtatgggtccaaagcctatgttaaacacccggcagacatacctgactacctcaagctctcctttcctgaggggtttaaatgggagagggtgatgaactttgaagatggaggcgtcgtgacagtaactcaggatagcagcctgcaagacggggagtttatttacaaggttaaattgcgcggaaccaactttcccagcgatggacccgtgatgcagaagaaaacaatgggctgggaagcatcatccgaaagaatgtatcccgaagatggcgcgttgaagggggaaatcaaacaaaggctcaagttgaaagatggagggcactatgacgctgaggtcaaaaccacgtacaaggctaaaaaaccggtacaactgcccggagcatataatgttaatattaagctggacatcaccagccacaatgaggattacacaatagtggaacagtatgaaagagccgagggaagacactcaactgggggcatggatgaactgtataaatgataa

SEQ ID NO: 16 - protein, 650 aa, synthetic construct
MGAQLTTFALAGAVRRMNTFQDQSGSSSNREPLLRCSDARRDLELAIGGVLRAEQQIKDNLREVKAQIHSCISRHLECLRSREVWLYEQVDLIYQLKEETLQQQAQQLYSLLGQFNCLTHQLECTQNKDLANQVSVCLERLGSLTLKPEDSTVLLFEADTITLRQTITTFGSLKTIQIPEHLMAHASSANIGPFLEKRGCISMPEQKSASGIVAVPFSEWLLGSKPASGYQAPYIPSTDPQDWLTQKQTLENSQTSSRACNFFNNVGGNLKGLENWLLKSEKSSYQKCNSHSTTSSFSIEMEKVGDQELPDQDEMDLSDWLVTPQESHKLRKPENGSRETSEKFKLLFQSYNVNDWLVKTDSCTNCQGNQPKGVEIENLGNLKCLNDHLEAKKPLSTPSMVTEDWLVQNHQDPCKVEEVCRANEPCTSFAECVCDENCEKEALYKWLLKKEGKDKNGMPVEPKPEPEKHKDSLNMWLCPRKEVIEQTKAPKAMTPSRIADSFQVIKNSPLSEWLIRPPYKEGSPKEVPGTEDRAGKQKFKSPMNTSWCSFNTADWVLPGKKMGNLSQLSSGEDKWLLRKKAQEVLLNSPLQEEHNFPPDHYGLPAVCDLFACMQLKVDKEKWLYRTPLQAYFKMNFQDVTVGNFQIPCGF

SEQ ID NO: 17 - DNA, 1953 bp, synthetic construct
  source 1..1953: mol_type = other DNA
atgggggcccagttgaccacttttgctctagctggagcagtgaggagaatgaataccttccaagaccagagtggcagctccagtaatagagaaccccttttgaggtgtagtgatgcacggagggacttggagcttgctattggtggagttctccgggctgaacagcaaattaaagataacttgcgagaggtcaaagctcagattcacagttgcataagccgtcacctggaatgtcttagaagccgtgaggtatggctgtatgaacaggtggaccttatttatcagcttaaagaggagacacttcaacagcaggctcagcagctctactcgttattgggccagttcaattgtcttactcatcaactggagtgtacccaaaacaaagatctagccaatcaagtctctgtgtgcctggagagactgggcagtttgacccttaagcctgaagattcaactgtcctgctctttgaagctgacacaattactctgcgccagaccatcaccacatttgggtctctcaaaaccattcaaattcctgagcacttgatggctcatgctagttcagcaaatattgggcccttcctggagaagagaggctgtatctccatgccagagcagaagtcagcatccggtattgtagctgtccctttcagcgaatggctccttggaagcaaacctgccagtggttatcaagctccttacatacccagcaccgacccccaggactggcttacccaaaagcagaccttggagaacagtcagacttcttccagagcctgcaatttcttcaataatgtcgggggaaacctaaagggcttagaaaactggctcctcaagagtgaaaaatcaagttatcaaaagtgtaacagccattccactactagttctttctccattgaaatggaaaaggttggagatcaagagcttcctgatcaagatgagatggacctatcagattggctagtgactccccaggaatcccataagctgcggaagcctgagaatggcagtcgtgaaaccagtgagaagtttaagctcttattccagtcctataatgtgaatgattggcttgtcaagactgactcctgtaccaactgtcagggaaaccagcccaaaggtgtggagattgaaaacctgggcaatctgaagtgcctgaatgaccacttggaggccaagaaaccattgtccacccccagcatggttacagaggattggcttgtccagaaccatcaggacccatgtaaggtagaggaggtgtgcagagccaatgagccctgcacaagctttgcagagtgtgtgtgtgatgagaattgtgagaaggaggctctgtataagtggcttctgaagaaagaaggaaaggataaaaatgggatgcctgtggaacccaaacctgagcctgagaagcataaagattccctgaatatgtggctctgtcctagaaaagaagtaatagaacaaactaaagcaccaaaggcaatgactccttctagaattgctgattccttccaagtcataaagaacagccccttgtcggagtggcttatcaggcccccatacaaagaaggaagtcccaaggaagtgcctggtactgaagacagagctggcaaacagaagtttaaaagccccatgaatacttcctggtgttcctttaacacagctgactgggtcctgccaggaaagaagatgggcaacctcagccagttatcttctggagaagacaagtggctgcttcgaaagaaggcccaggaagtattacttaattcacctctacaggaggaacataacttccccccagaccattatggcctccctgcagtttgtgatctctttgcctgtatgcagcttaaagttgataaagagaagtggttatatcgaactcctctacaggcatacttcaaaatgaactttcaagatgtaaccgttgggaattttcagatcccatgtggattctag

SEQ ID NO: 18 - DNA, 4047 bp, synthetic construct
  source 1..4047: mol_type = other DNA
caactttgtatagaaaagttggggttgcgccttttccaaggcagccctgggtttgcgcagggacgcggctgctctgggcgtggttccgggaaacgcagcggcgccgaccctgggtctcgcacattcttcacgtccgttcgcagcgtcacccggatcttcgccgctacccttgtgggccccccggcgacgcttcctgctccgcccctaagtcgggaaggttccttgcggttcgcggcgtgccggacgtgacaaacggaagccgcacgtctcactagtaccctcgcagacggacagcgccagggagcaatggcagcgcgccgaccgcgatgggctgtggccaatagcggctgctcagcagggcgcgccgagagcagcggccgggaaggggcggtgcgggaggcggggtgtggggcggtagtgtgggccctgttcctgcccgcgcggtgttccgcattctgcaagcctccggagcgcacgtcggcagtcggctccctcgttgaccgaatcaccgacctctctccccagggctagcgccaccatggcgccctttcctgaagaagtggacgtcttcaccgccccacactggcggatgaagcagctggtggggctctactgcgacaagctttctaaaaccaatttttccaacaacaacgatttccgtgctcttctgcagtctttgtatgctactttcaaggagttcaaaatgcatgagcagattgaaaatgaatacattattggtttgcttcaacaacgcagccagaccatttataatgtacattctgacaataaactctccgagatgcttagcctctttgaaaagggactgaagaatgttaagaatgaatatgaacagttaaattatgcaaaacaactgaaagagagattggaggcttttacaagagattttcttcctcacatgaaagaggaagaggaggtttttcagcccatgttaatggaatattttacctatgaagagcttaaggatattaaaaagaaagtgattgcacaacactgctctggcggcggctctagagtgtctaagggcgaagagctgattaaggagaacatgcacatgaagctgtacatggagggcaccgtggacaaccatcacttcaagtgcacatccgagggcgaaggcaagccctacgagggcacccagaccatgagaatcaaggtggtcgagggcggccctctccccttcgccttcgacatcctggctactagcttcctctacggcagcaagaccttcatcaaccacacccagggcatccccgacttcttcaagcagtccttccctgagggcttcacatgggagagagtcaccacatacgaagacgggggcgtgctgaccgctacccaggacaccagcctccaggacggctgcctcatctacaacgtcaagatcagaggggtgaacttcacatccaacggccctgtgatgcagaagaaaacactcggctgggaggccttcaccgagacgctgtaccccgctgacggcggcctggaaggcagaaacgacatggccctgaagctcgtgggcgggagccatctgatcgcaaacgccaagaccacatatagatccaagaaacccgctaagaacctcaagatgcctggcgtctactatgtggactacagactggaaagaatcaaggaggccaacaacgagacctacgtcgagcagcacgaggtggcagtggccagatactgcgacctccctagcaaactggggcacaagcttaattaagaattcacccagctttcttgtacaaagtggtgatggccggccgcttcgagcagacatgataagatacattgatgagtttggacaaaccacaactagaatgcagtgaaaaaaatgctttatttgtgaaatttgtgatgctattgctttatttgtaaccattataagctgcaataaacaagttaacaacaacaattgcattcattttatgtttcaggttcagggggaggtgtgggaggttttttaaagcaagtaaaacctctacaaatgtggtagcggccgcggcgctcttccgcttcctcgctcactgactcgctgcgctcggtcgttcggctgcggcgagcggtatcagctcactcaaaggcggtaatacggttatccacagaatcaggggataacgcaggaaagaacatgtgagcaaaaggccagcaaaaggccaggaaccgtaaaaaggccgcgttgctggcgtttttccataggctccgcccccctgacgagcatcacaaaaatcgacgctcaagtcagaggtggcgaaacccgacaggactataaagataccaggcgtttccccctggaagctccctcgtgcgctctcctgttccgaccctgccgcttaccggatacctgtccgcctttctctcttcgggaagcgtggcgctttctcatagctcacgctgtaggtatctcagttcggtgtaggtcgttcgctccaagctgggctgtgtgcacgaaccccccgttcagcccgaccgctgcgccttatccggtaactatcgtcttgagtccaacccggtaagacacgacttatcgccactggcagcagccactggtaacaggattagcagagcgaggtatgtaggcggtgctacagagttcttgaagtggtggcctaactacggctacactagaagaacagtatttggtatctgcgctctgctgaagccagttaccttcggaaaaagagttggtagctcttgatccggcaaacaaaccaccgctggtagcggtggtttttttgtttgcaagcagcagattacgcgcagaaaaaaaggatctcaagaagatcctttgatcttttctacggggtctgacgctcagtggaacgaaaactcacgttaagggattttggtcatgagattatcaaaaaggatcttcacctagatccttttaaattaaaaatgaagttttaaatcaatctaaagtatatatgagtaaacttggtctgacagttaccaatgcttaatcagtgaggcacctatctcagcgatctgtctatttcgttcatccatagttgcctgactccccgtcgtgtagataactacgatacgggagggcttaccatctggccccagtgctgcaatgataccgcgagacccacgctcaccggctccagatttatcagcaataaaccagccagccggaagggccgagcgcagaagtggtcctgcaactttatccgcctccatccagtctattaattgttgccgggaagctagagtaagtagttcgccagttaatagtttgcgcaacgttgttgccattgctacaggcatcgtggtgtcacgctcgtcgtttggtatggcttcattcagctccggttcccaacgatcaaggcgagttacatgatcccccatgttgtgcaaaaaagcggttagctccttcggtcctccgatcgttgtcagaagtaagttggccgcagtgttatcactcatggttatggcagcactgcataattctcttactgtcatgccatccgtaagatgcttttctgtgactggtgagtactcaaccaagtcattctgagaatagtgtatgcggcgaccgagttgctcttgcccggcgtcaatacgggataataccgcgccacatagcagaactttaaaagtgctcatcattggaaaacgttcttcggggcgaaaactctcaaggatcttaccgctgttgagatccagttcgatgtaacccactcgtgcacccaactgatcttcagcatcttttactttcaccagcgtttctgggtgagcaaaaacaggaaggcaaaatgccgcaaaaaagggaataagggcgacacggaaatgttgaatactcatactcttcctttttcaatattattgaagcatttatcagggttattgtctcatgagcggatacatatttgaatgtatttagaaaaataaacaaataggggttccgcgcacatttccccgaaaagtgccacctgacgtctaagaaaccattattatcatgacattaacctataaaaataggcgtatcacgaggccctttcgtcggcgcgccgcggccgc

SEQ ID NO: 19 - DNA, 4812 bp, synthetic construct
  source 1..4812: mol_type = other DNA
caactttgtatagaaaagttgggatccgggttgcgccttttccaaggcagccctgggtttgcgcagggacgcggctgctctgggcgtggttccgggaaacgcagcggcgccgaccctgggtctcgcacattcttcacgtccgttcgcagcgtcacccggatcttcgccgctacccttgtgggccccccggcgacgcttcctgctccgcccctaagtcgggaaggttccttgcggttcgcggcgtgccggacgtgacaaacggaagccgcacgtctcactagtaccctcgcagacggacagcgccagggagcaatggcagcgcgccgaccgcgatgggctgtggccaatagcggctgctcagcagggcgcgccgagagcagcggccgggaaggggcggtgcgggaggcggggtgtggggcggtagtgtgggccctgttcctgcccgcgcggtgttccgcattctgcaagcctccggagcgcacgtcggcagtcggctccctcgttgaccgaatcaccgacctctctccccagggccaccatggcgccctttcctgaagaagtggacgtcttcaccgccccacactggcggatgaagcagctggtggggctctactgcgacaagctttctaaaaccaatttttccaacaacaacgatttccgtgctcttctgcagtctttgtatgctactttcaaggagttcaaaatgcatgagcagattgaaaatgaatacattattggtttgcttcaacaacgcagccagaccatttataatgtacattctgacaataaactctccgagatgcttagcctctttgaaaagggactgaagaatgttaagaatgaatatgaacagttaaattatgcaaaacaactgaaagagagattggaggcttttacaagagattttcttcctcacatgaaagaggaagaggaggtttttcagcccatgttaatggaatattttacctatgaagagcttaaggatattaaaaagaaagtgattgcacaacactgctctggcggcggcgtgagtaagggggaggaagataacatggcctcacttccagcgactcacgaacttcacatttttgggtccatcaatggcgtggatttcgatatggtagggcaagggactggcaaccctaacgacggttacgaagaactcaatctgaaatcaacgaaaggggatttgcaattttccccatggatactcgtcccccatataggctatggattccaccaatatctgccgtatccagacggaatgtctccgtttcaagccgcaatggtagacggtagcggttaccaggtccaccggacgatgcaattcgaagatggggcctccctgacagtaaattatagatatacctatgaagggagtcacataaagggagaagctcaggtcaaaggaacgggtttcccggctgacggaccggtgatgaccaattcactgaccgccgccgattggtgccgctctaaaaaaacttacccaaatgataagactatcatttcaacttttaaatggagttacactacggggaatggtaagaggtacaggtcaacagccaggacaacttacacatttgccaagccaatggcggcgaactatttgaaaaatcagccaatgtacgttttccgaaaaaccgaattgaaacattctaagaccgagcttaatttcaaggaatggcaaaaagcatttacggatgtgatggggatggatgagctttacaagggtaccggaagcggagagggcaggggaagtcttctaacatgcggggacgtggaggaaaatcccggccccatggtctccaaaggagaggaagacaatatggccattatcaaagagtttatgcgatttaaagtgcacatggagggaagcgtcaacgggcatgagtttgagattgagggggaaggagagggaagaccttatgaagggacccagactgccaaactgaaagtcaccaagggcggacccctgccatttgcttgggacattctgagcccacaattcatgtatgggtccaaagcctatgttaaacacccggcagacatacctgactacctcaagctctcctttcctgaggggtttaaatgggagagggtgatgaactttgaagatggaggcgtcgtgacagtaactcaggatagcagcctgcaagacggggagtttatttacaaggttaaattgcgcggaaccaactttcccagcgatggacccgtgatgcagaagaaaacaatgggctgggaagcatcatccgaaagaatgtatcccgaagatggcgcgttgaagggggaaatcaaacaaaggctcaagttgaaagatggagggcactatgacgctgaggtcaaaaccacgtacaaggctaaaaaaccggtacaactgcccggagcatataatgttaatattaagctggacatcaccagccacaatgaggattacacaatagtggaacagtatgaaagagccgagggaagacactcaactgggggcatggatgaactgtataaatgataaacccagctttcttgtacaaagtggtgatggccggccgcttcgagcagacatgataagatacattgatgagtttggacaaaccacaactagaatgcagtgaaaaaaatgctttatttgtgaaatttgtgatgctattgctttatttgtaaccattataagctgcaataaacaagttaacaacaacaattgcattcattttatgtttcaggttcagggggaggtgtgggaggttttttaaagcaagtaaaacctctacaaatgtggtagcggccgcggcgctcttccgcttcctcgctcactgactcgctgcgctcggtcgttcggctgcggcgagcggtatcagctcactcaaaggcggtaatacggttatccacagaatcaggggataacgcaggaaagaacatgtgagcaaaaggccagcaaaaggccaggaaccgtaaaaaggccgcgttgctggcgtttttccataggctccgcccccctgacgagcatcacaaaaatcgacgctcaagtcagaggtggcgaaacccgacaggactataaagataccaggcgtttccccctggaagctccctcgtgcgctctcctgttccgaccctgccgcttaccggatacctgtccgcctttctctcttcgggaagcgtggcgctttctcatagctcacgctgtaggtatctcagttcggtgtaggtcgttcgctccaagctgggctgtgtgcacgaaccccccgttcagcccgaccgctgcgccttatccggtaactatcgtcttgagtccaacccggtaagacacgacttatcgccactggcagcagccactggtaacaggattagcagagcgaggtatgtaggcggtgctacagagttcttgaagtggtggcctaactacggctacactagaagaacagtatttggtatctgcgctctgctgaagccagttaccttcggaaaaagagttggtagctcttgatccggcaaacaaaccaccgctggtagcggtggtttttttgtttgcaagcagcagattacgcgcagaaaaaaaggatctcaagaagatcctttgatcttttctacggggtctgacgctcagtggaacgaaaactcacgttaagggattttggtcatgagattatcaaaaaggatcttcacctagatccttttaaattaaaaatgaagttttaaatcaatctaaagtatatatgagtaaacttggtctgacagttaccaatgcttaatcagtgaggcacctatctcagcgatctgtctatttcgttcatccatagttgcctgactccccgtcgtgtagataactacgatacgggagggcttaccatctggccccagtgctgcaatgataccgcgagacccacgctcaccggctccagatttatcagcaataaaccagccagccggaagggccgagcgcagaagtggtcctgcaactttatccgcctccatccagtctattaattgttgccgggaagctagagtaagtagttcgccagttaatagtttgcgcaacgttgttgccattgctacaggcatcgtggtgtcacgctcgtcgtttggtatggcttcattcagctccggttcccaacgatcaaggcgagttacatgatcccccatgttgtgcaaaaaagcggttagctccttcggtcctccgatcgttgtcagaagtaagttggccgcagtgttatcactcatggttatggcagcactgcataattctcttactgtcatgccatccgtaagatgcttttctgtgactggtgagtactcaaccaagtcattctgagaatagtgtatgcggcgaccgagttgctcttgcccggcgtcaatacgggataataccgcgccacatagcagaactttaaaagtgctcatcattggaaaacgttcttcggggcgaaaactctcaaggatcttaccgctgttgagatccagttcgatgtaacccactcgtgcacccaactgatcttcagcatcttttactttcaccagcgtttctgggtgagcaaaaacaggaaggcaaaatgccgcaaaaaagggaataagggcgacacggaaatgttgaatactcatactcttcctttttcaatattattgaagcatttatcagggttattgtctcatgagcggatacatatttgaatgtatttagaaaaataaacaaataggggttccgcgcacatttccccgaaaagtgccacctgacgtctaagaaaccattattatcatgacattaacctataaaaataggcgtatcacgaggccctttcgtcggcgcgccgcggccgc

SEQ ID NO: 20 - DNA, 22 bp, synthetic construct
  source 1..22: mol_type = other DNA
gatcgccctacgtgctgtctca

SEQ ID NO: 21 - DNA, 176 bp, synthetic construct
  source 1..176: mol_type = other DNA
gatcgccctacgtgctgtctcagatcgccctacgtgctgtctcagatcgccctacgtgctgtctcagatcgccctacgtgctgtctcagatcgccctacgtgctgtctcagatcgccctacgtgctgtctcagatcgccctacgtgctgtctcagatcgccctacgtgctgtctca

SEQ ID NO: 22 - DNA, 33 bp, synthetic construct
  source 1..33: mol_type = other DNA
tgtctcttgcttcaacagtgtttggacggaaca

SEQ ID NO: 23 - DNA, 1496 bp, synthetic construct
  source 1..1496: mol_type = other DNA
atgtgatacccatagcttccatgagaacagcagggtagtctggtttctagacttgtgctgatcgtgctaaattttcagtagggctacaaaacctgatgttaaaattccatcccatcatcttggtactactagatgtctttaggcagcagcttttaatacagggtagataacctgtacttcaagttaaagtgaataaccacttaaaaaatgtccatgatggaatattcccctatctctagaattttaagtgctttgtaatgggaactgcctctttcctgttgttgttaatgaaaatgtcagaaaccagttatgtgaatgatctctctgaatcctaagggctggtctctgctgaaggttgtaagtggtcgcttactttgagtgatcctccaacttcatttgatgctaaataggagataccaggttgaaagaccttctccaaatgagatctaagcctttccataaggaatgtagctggtttcctcattcctgaaagaaacagttaactttcagaagagatgggcttgttttcttgccaatgaggtctgaaatggaggtccttctgctggataaaatgaggttcaactgttgattgcaggaataaggccttaatatgttaacctcagtgtcatttatgaaaagaggggaccagaagccaaagacttagtatattttcttttcctctgtcccttcccccataagcctccatttagttctttgttatttttgtttcttccaaagcacattgaaagagaaccagtttcaggtgtttagttgcagactcagtttgtcagactttaaagaataatatgctgccaaattttggccaaagtgttaatcttaggggagagctttctgtccttttggcactgagatatttattgtttatttatcagtgacagagttcactataaatggtgtttttttaatagaatataattatcggaagcagtgccttccataattatgacagttatactgtcggttttttttaaataaaagcagcatctgctaataaaacccaacagatactggaagttttgcatttatggtcaacacttaagggttttagaaaacagccgtcagccaaatgtaattgaataaagttgaagctaagatttagagatgaattaaatttaattaggggttgctaagaagcgagcactgaccagataagaatgctggttttcctaaatgcagtgaattgtgaccaagttataaatcaatgtcacttaaaggctgtggtagtactcctgcaaaattttatagctcagtttatccaaggtgtaactctaattcccattttgcaaaatttccagtacctttgtcacaatcctaacacattatcgggagcagtgtcttccataatgtataaagaacaaggtagtttttacctaccacagtgtctgtatcggagacagtgatctccatatgttacactaagggtgtaagtaattatcgggaacagtgtttcccataattttcttcatgcaatgaca

SEQ ID NO: 24 - DNA, 2428 bp, synthetic construct
  source 1..2428: mol_type = other DNA
gatcgccctacgtgctgtctcagatcgccctacgtgctgtctcagatcgccctacgtgctgtctcagatcgccctacgtgctgtctcagatcgccctacgtgctgtctcagatcgccctacgtgctgtctcagatcgccctacgtgctgtctcagatcgccctacgtgctgtctcacaagtttgtacaaaaaagcaggctgccaccgtcgacatggtgagtaagggggaggaagataacatggcctcacttccagcgactcacgaacttcacatttttgggtccatcaatggcgtggatttcgatatggtagggcaagggactggcaaccctaacgacggttacgaagaactcaatctgaaatcaacgaaaggggatttgcaattttccccatggatactcgtcccccatataggctatggattccaccaatatctgccgtatccagacggaatgtctccgtttcaagccgcaatggtagacggtagcggttaccaggtccaccggacgatgcaattcgaagatggggcctccctgacagtaaattatagatatacctatgaagggagtcacataaagggagaagctcaggtcaaaggaacgggtttcccggctgacggaccggtgatgaccaattcactgaccgccgccgattggtgccgctctaaaaaaacttacccaaatgataagactatcatttcaacttttaaatggagttacactacggggaatggtaagaggtacaggtcaacagccaggacaacttacacatttgccaagccaatggcggcgaactatttgaaaaatcagccaatgtacgttttccgaaaaaccgaattgaaacattctaagaccgagcttaatttcaaggaatggcaaaaagcatttacggatgtgatggggatggatgagctttacaagtaataaggtaccatgtgatacccatagcttccatgagaacagcagggtagtctggtttctagacttgtgctgatcgtgctaaattttcagtagggctacaaaacctgatgttaaaattccatcccatcatcttggtactactagatgtctttaggcagcagcttttaatacagggtagataacctgtacttcaagttaaagtgaataaccacttaaaaaatgtccatgatggaatattcccctatctctagaattttaagtgctttgtaatgggaactgcctctttcctgttgttgttaatgaaaatgtcagaaaccagttatgtgaatgatctctctgaatcctaagggctggtctctgctgaaggttgtaagtggtcgcttactttgagtgatcctccaacttcatttgatgctaaataggagataccaggttgaaagaccttctccaaatgagatctaagcctttccataaggaatgtagctggtttcctcattcctgaaagaaacagttaactttcagaagagatgggcttgttttcttgccaatgaggtctgaaatggaggtccttctgctggataaaatgaggttcaactgttgattgcaggaataaggccttaatatgttaacctcagtgtcatttatgaaaagaggggaccagaagccaaagacttagtatattttcttttcctctgtcccttcccccataagcctccatttagttctttgttatttttgtttcttccaaagcacattgaaagagaaccagtttcaggtgtttagttgcagactcagtttgtcagactttaaagaataatatgctgccaaattttggccaaagtgttaatcttaggggagagctttctgtccttttggcactgagatatttattgtttatttatcagtgacagagttcactataaatggtgtttttttaatagaatataattatcggaagcagtgccttccataattatgacagttatactgtcggttttttttaaataaaagcagcatctgctaataaaacccaacagatactggaagttttgcatttatggtcaacacttaagggttttagaaaacagccgtcagccaaatgtaattgaataaagttgaagctaagatttagagatgaattaaatttaattaggggttgctaagaagcgagcactgaccagataagaatgctggttttcctaaatgcagtgaattgtgaccaagttataaatcaatgtcacttaaaggctgtggtagtactcctgcaaaattttatagctcagtttatccaaggtgtaactctaattcccattttgcaaaatttccagtacctttgtcacaatcctaacacattatcgggagcagtgtcttccataatgtataaagaacaaggtagtttttacctaccacagtgtctgtatcggagacagtgatctccatatgttacactaagggtgtaagtaattatcgggaacagtgtttcccataattttcttcatgcaatgaca

SEQ ID NO: 25 - DNA, 225 bp, synthetic construct
  source 1..225: mol_type = other DNA
ctgtgccttctagttgccagccatctgttgtttgcccctcccccgtgccttccttgaccctggaaggtgccactcccactgtcctttcctaataaaatgaggaaattgcatcgcattgtctgagtaggtgtcattctattctggggggtggggtggggcaggacagcaagggggaggattgggaagacaatagcaggcatgctggggatgcggtgggctctatgg

SEQ ID NO: 26 - DNA, 48 bp, synthetic construct
  source 1..48: mol_type = other DNA
gtagcataaccccttggggcctctaaacgggtcttgaggggttttttg

SEQ ID NO: 27 - DNA, 137 bp, synthetic construct
  source 1..137: mol_type = other DNA
gcattggcgcagaaaaaaatgcctgatgcgacgctgcgcgtcttatactcccacatatgccagattcagcaacggatacggcttccccaacttgcccacttccatacgtgtcctccttaccagaaatttatccttaa

SEQ ID NO: 28 - DNA, 1935 bp, synthetic construct
  source 1..1935: mol_type = other DNA
ttgcgccttttccaaggcagccctgggtttgcgcagggacgcggctgctctgggcgtggttccgggaaacgcagcggcgccgaccctgggtctcgcacattcttcacgtccgttcgcagcgtcacccggatcttcgccgctacccttgtgggccccccggcgacgcttcctgctccgcccctaagtcgggaaggttccttgcggttcgcggcgtgccggacgtgacaaacggaagccgcacgtctcactagtaccctcgcagacggacagcgccagggagcaatggcagcgcgccgaccgcgatgggctgtggccaatagcggctgctcagcagggcgcgccgagagcagcggccgggaaggggcggtgcgggaggcggggtgtggggcggtagtgtgggccctgttcctgcccgcgcggtgttccgcattctgcaagcctccggagcgcacgtcggcagtcggctccctcgttgaccgaatcaccgacctctctccccaggcaagtttgtacaaaaaagcaggctgccacctgtctcttgcttcaacagtgtttggacggaacagctagcatggtctccaaaggagaggaagacaatatggccattatcaaagagtttatgcgatttaaagtgcacatggagggaagcgtcaacgggcatgagtttgagattgagggggaaggagagggaagaccttatgaagggacccagactgccaaactgaaagtcaccaagggcggacccctgccatttgcttgggacattctgagcccacaattcatgtatgggtccaaagcctatgttaaacacccggcagacatacctgactacctcaagctctcctttcctgaggggtttaaatgggagagggtgatgaactttgaagatggaggcgtcgtgacagtaactcaggatagcagcctgcaagacggggagtttatttacaaggttaaattgcgcggaaccaactttcccagcgatggacccgtgatgcagaagaaaacaatgggctgggaagcatcatccgaaagaatgtatcccgaagatggcgcgttgaagggggaaatcaaacaaaggctcaagttgaaagatggagggcactatgacgctgaggtcaaaaccacgtacaaggctaaaaaaccggtacaactgcccggagcatataatgttaatattaagctggacatcaccagccacaatgaggattacacaatagtggaacagtatgaaagagccgagggaagacactcaactgggggcatggatgaactgtataaatgagaattcctgtgccttctagttgccagccatctgttgtttgcccctcccccgtgccttccttgaccctggaaggtgccactcccactgtcctttcctaataaaatgaggaaattgcatcgcattgtctgagtaggtgtcattctattctggggggtggggtggggcaggacagcaagggggaggattgggaagacaatagcaggcatgctggggatgcggtgggctctatgggcattggcgcagaaaaaaacaacaacaattgcattcattttatgtttcaggttcagggggaggtgtgggaggttttttaaagcaagtaaaacctctacaaatgtggtattggcccatctctatcggtatcgtagcataaccccttggggcctctaaacgggtcttgaggggttttttgtgcccctcgggccggattgctatctaccggcattggcgcagaaaaaaatgcctgatgcgacgctgcgcgtcttatactcccacatatgccagattcagcaacggatacggcttccccaacttgcccacttccatacgtgtcctccttaccagaaatttatccttaaggtcgtcagctatcctgcaggatagtaatcaattacggggtcattagttcatagcccatatatggagttccgggatcc

SEQ ID NO: 29 - DNA, 8813 bp, synthetic construct
  source 1..8813: mol_type = other DNA
gacggatcgggagatctttgcgccttttccaaggcagccctgggtttgcgcagggacgcggctgctctgggcgtggttccgggaaacgcagcggcgccgaccctgggtctcgcacattcttcacgtccgttcgcagcgtcacccggatcttcgccgctacccttgtgggccccccggcgacgcttcctgctccgcccctaagtcgggaaggttccttgcggttcgcggcgtgccggacgtgacaaacggaagccgcacgtctcactagtaccctcgcagacggacagcgccagggagcaatggcagcgcgccgaccgcgatgggctgtggccaatagcggctgctcagcagggcgcgccgagagcagcggccgggaaggggcggtgcgggaggcggggtgtggggcggtagtgtgggccctgttcctgcccgcgcggtgttccgcattctgcaagcctccggagcgcacgtcggcagtcggctccctcgttgaccgaatcaccgacctctctccccaggcaagtttgtacaaaaaagcaggctgccacctgtctcttgcttcaacagtgtttggacggaacagctagcatggtctccaaaggagaggaagacaatatggccattatcaaagagtttatgcgatttaaagtgcacatggagggaagcgtcaacgggcatgagtttgagattgagggggaaggagagggaagaccttatgaagggacccagactgccaaactgaaagtcaccaagggcggacccctgccatttgcttgggacattctgagcccacaattcatgtatgggtccaaagcctatgttaaacacccggcagacatacctgactacctcaagctctcctttcctgaggggtttaaatgggagagggtgatgaactttgaagatggaggcgtcgtgacagtaactcaggatagcagcctgcaagacggggagtttatttacaaggttaaattgcgcggaaccaactttcccagcgatggacccgtgatgcagaagaaaacaatgggctgggaagcatcatccgaaagaatgtatcccgaagatggcgcgttgaagggggaaatcaaacaaaggctcaagttgaaagatggagggcactatgacgctgaggtcaaaaccacgtacaaggctaaaaaaccggtacaactgcccggagcatataatgttaatattaagctggacatcaccagccacaatgaggattacacaatagtggaacagtatgaaagagccgagggaagacactcaactgggggcatggatgaactgtataaatgagaattcctgtgccttctagttgccagccatctgttgtttgcccctcccccgtgccttccttgaccctggaaggtgccactcccactgtcctttcctaataaaatgaggaaattgcatcgcattgtctgagtaggtgtcattctattctggggggtggggtggggcaggacagcaagggggaggattgggaagacaatagcaggcatgctggggatgcggtgggctctatgggcattggcgcagaaaaaaacaacaacaattgcattcattttatgtttcaggttcagggggaggtgtgggaggttttttaaagcaagtaaaacctctacaaatgtggtattggcccatctctatcggtatcgtagcataaccccttggggcctctaaacgggtcttgaggggttttttgtgcccctcgggccggattgctatctaccggcattggcgcagaaaaaaatgcctgatgcgacgctgcgcgtcttatactcccacatatgccagattcagcaacggatacggcttccccaacttgcccacttccatacgtgtcctccttaccagaaatttatccttaaggtcgtcagctatcctgcaggatagtaatcaattacggggtcattagttcatagcccatatatggagttccgggatccgatcgccctacgtgctgtctcagatcgccctacgtgctgtctcagatcgccctacgtgctgtctcagatcgccctacgtgctgtctcagatcgccctacgtgctgtctcagatcgccctacgtgctgtctcagatcgccctacgtgctgtctcagatcgccctacgtgctgtctcacaagtttgtacaaaaaagcaggctgccaccgtcgacatggtgagtaagggggaggaagataacatggcctcacttccagcgactcacgaacttcacatttttgggtccatcaatggcgtggatttcgatatggtagggcaagggactggcaaccctaacgacggttacgaagaactcaatctgaaatcaacgaaaggggatttgcaattttccccatggatactcgtcccccatataggctatggattccaccaatatctgccgtatccagacggaatgtctccgtttcaagccgcaatggtagacggtagcggttaccaggtccaccggacgatgcaattcgaagatggggcctccctgacagtaaattatagatatacctatgaagggagtcacataaagggagaagctcaggtcaaaggaacgggtttcccggctgacggaccggtgatgaccaattcactgaccgccgccgattggtgccgctctaaaaaaacttacccaaatgataagactatcatttcaacttttaaatggagttacactacggggaatggtaagaggtacaggtcaacagccaggacaacttacacatttgccaagccaatggcggcgaactatttgaaaaatcagccaatgtacgttttccgaaaaaccgaattgaaacattctaagaccgagcttaatttcaaggaatggcaaaaagcatttacggatgtgatggggatggatgagctttacaagtaataaggtaccatgtgatacccatagcttccatgagaacagcagggtagtctggtttctagacttgtgctgatcgtgctaaattttcagtagggctacaaaacctgatgttaaaattccatcccatcatcttggtactactagatgtctttaggcagcagcttttaatacagggtagataacctgtacttcaagttaaagtgaataaccacttaaaaaatgtccatgatggaatattcccctatctctagaattttaagtgctttgtaatgggaactgcctctttcctgttgttgttaatgaaaatgtcagaaaccagttatgtgaatgatctctctgaatcctaagggctggtctctgctgaaggttgtaagtggtcgcttactttgagtgatcctccaacttcatttgatgctaaataggagataccaggttgaaagaccttctccaaatgagatctaagcctttccataaggaatgtagctggtttcctcattcctgaaagaaacagttaactttcagaagagatgggcttgttttcttgccaatgaggtctgaaatggaggtccttctgctggataaaatgaggttcaactgttgattgcaggaataaggccttaatatgttaacctcagtgtcatttatgaaaagaggggaccagaagccaaagacttagtatattttcttttcctctgtcccttcccccataagcctccatttagttctttgttatttttgtttcttccaaagcacattgaaagagaaccagtttcaggtgtttagttgcagactcagtttgtcagactttaaagaataatatgctgccaaattttggccaaagtgttaatcttaggggagagctttctgtccttttggcactgagatatttattgtttatttatcagtgacagagttcactataaatggtgtttttttaatagaatataattatcggaagcagtgccttccataattatgacagttatactgtcggttttttttaaataaaagcagcatctgctaataaaacccaacagatactggaagttttgcatttatggtcaacacttaagggttttagaaaacagccgtcagccaaatgtaattgaataaagttgaagctaagatttagagatgaattaaatttaattaggggttgctaagaagcgagcactgaccagataagaatgctggttttcctaaatgcagtgaattgtgaccaagttataaatcaatgtcacttaaaggctgtggtagtactcctgcaaaattttatagctcagtttatccaaggtgtaactctaattcccattttgcaaaatttccagtacctttgtcacaatcctaacacattatcgggagcagtgtcttccataatgtataaagaacaaggtagtttttacctaccacagtgtctgtatcggagacagtgatctccatatgttacactaagggtgtaagtaattatcgggaacagtgtttcccataattttcttcatgcaatgacaaagcttaagtttaaaccgctgatcagcctcgactgtgccttctagttgccagccatctgttgtttgcccctcccccgtgccttccttgaccctggaaggtgccactcccactgtcctttcctaataaaatgaggaaattgcatcgcattgtctgagtaggtgtcattctattctggggggtggggtggggcaggacagcaagggggaggattgggaagacaatagcaggcatgctggggatgcggtgggctctatggcttctgaggcggaaagaaccagctggggctctagggggtatccccacgcgccctgtagcggcgcattaagcgcggcgggtgtggtggttacgcgcagcgtgaccgctacacttgccagcgccctagcgcccgctcctttcgctttcttcccttcctttctcgccacgttcgccggctttccccgtcaagctctaaatcgggggctccctttagggttccgatttagtgctttacggcacctcgaccccaaaaaacttgattagggtgatggttcacgtagtgggccatcgccctgatagacggtttttcgccctttgacgttggagtccacgttctttaatagtggactcttgttccaaactggaacaacactcaaccctatctcggtctattcttttgatttataagggattttgccgatttcggcctattggttaaaaaatgagctgatttaacaaaaatttaacgcgaattaattctgtggaatgtgtgtcagttagggtgtggaaagtccccaggctccccagcaggcagaagtatgcaaagcatgcatctcaattagtcagcaaccaggtgtggaaagtccccaggctccccagcaggcagaagtatgcaaagcatgcatctcaattagtcagcaaccatagtcccgcccctaactccgcccatcccgcccctaactccgcccagttccgcccattctccgccccatggctgactaattttttttatttatgcagaggccgaggccgcctctgcctctgagctattccagaagtagtgaggaggcttttttggaggcctaggcttttgcaaaaagctcccgggagcttgtatatccattttcggatctgatcaagagacaggatgaggatcgtttcgcatgattgaacaagatggattgcacgcaggttctccggccgcttgggtggagaggctattcggctatgactgggcacaacagacaatcggctgctctgatgccgccgtgttccggctgtcagcgcaggggcgcccggttctttttgtcaagaccgacctgtccggtgccctgaatgaactgcaggacgaggcagcgcggctatcgtggctggccacgacgggcgttccttgcgcagctgtgctcgacgttgtcactgaagcgggaagggactggctgctattgggcgaagtgccggggcaggatctcctgtcatctcaccttgctcctgccgagaaagtatccatcatggctgatgcaatgcggcggctgcatacgcttgatccggctacctgcccattcgaccaccaagcgaaacatcgcatcgagcgagcacgtactcggatggaagccggtcttgtcgatcaggatgatctggacgaagagcatcaggggctcgcgccagccgaactgttcgccaggctcaaggcgcgcatgcccgacggcgaggatctcgtcgtgacccatggcgatgcctgcttgccgaatatcatggtggaaaatggccgcttttctggattcatcgactgtggccggctgggtgtggcggaccgctatcaggacatagcgttggctacccgtgatattgctgaagagcttggcggcgaatgggctgaccgcttcctcgtgctttacggtatcgccgctcccgattcgcagcgcatcgccttctatcgccttcttgacgagttcttctgagcgggactctggggttcgaaatgaccgaccaagcgacgcccaacctgccatcacgagatttcgattccaccgccgccttctatgaaaggttgggcttcggaatcgttttccgggacgccggctggatgatcctccagcgcggggatctcatgctggagttcttcgcccaccccaacttgtttattgcagcttataatggttacaaataaagcaatagcatcacaaatttcacaaataaagcatttttttcactgcattctagttgtggtttgtccaaactcatcaatgtatcttatcatgtctgtataccgtcgacctctagctagagcttggcgtaatcatggtcatagctgtttcctgtgtgaaattgttatccgctcacaattccacacaacatacgagccggaagcataaagtgtaaagcctggggtgcctaatgagtgagctaactcacattaattgcgttgcgctcactgcccgctttccagtcgggaaacctgtcgtgccagctgcattaatgaatcggccaacgcgcggggagaggcggtttgcgtattgggcgctcttccgcttcctcgctcactgactcgctgcgctcggtcgttcggctgcggcgagcggtatcagctcactcaaaggcggtaatacggttatccacagaatcaggggataacgcaggaaagaacatgtgagcaaaaggccagcaaaaggccaggaaccgtaaaaaggccgcgttgctggcgtttttccataggctccgcccccctgacgagcatcacaaaaatcgacgctcaagtcagaggtggcgaaacccgacaggactataaagataccaggcgtttccccctggaagctccctcgtgcgctctcctgttccgaccctgccgcttaccggatacctgtccgcctttctcccttcgggaagcgtggcgctttctcatagctcacgctgtaggtatctcagttcggtgtaggtcgttcgctccaagctgggctgtgtgcacgaaccccccgttcagcccgaccgctgcgccttatccggtaactatcgtcttgagtccaacccggtaagacacgacttatcgccactggcagcagccactggtaacaggattagcagagcgaggtatgtaggcggtgctacagagttcttgaagtggtggcctaactacggctacactagaagaacagtatttggtatctgcgctctgctgaagccagttaccttcggaaaaagagttggtagctcttgatccggcaaacaaaccaccgctggtagcggtttttttgtttgcaagcagcagattacgcgcagaaaaaaaggatctcaagaagatcctttgatcttttctacggggtctgacgctcagtggaacgaaaactcacgttaagggattttggtcatgagattatcaaaaaggatcttcacctagatccttttaaattaaaaatgaagttttaaatcaatctaaagtatatatgagtaaacttggtctgacagttaccaatgcttaatcagtgaggcacctatctcagcgatctgtctatttcgttcatccatagttgcctgactccccgtcgtgtagataactacgatacgggagggcttaccatctggccccagtgctgcaatgataccgcgagacccacgctcaccggctccagatttatcagcaataaaccagccagccggaagggccgagcgcagaagtggtcctgcaactttatccgcctccatccagtctattaattgttgccgggaagctagagtaagtagttcgccagttaatagtttgcgcaacgttgttgccattgctacaggcatcgtggtgtcacgctcgtcgtttggtatggcttcattcagctccggttcccaacgatcaaggcgagttacatgatcccccatgttgtgcaaaaaagcggttagctccttcggtcctccgatcgttgtcagaagtaagttggccgcagtgttatcactcatggttatggcagcactgcataattctcttactgtcatgccatccgtaagatgcttttctgtgactggtgagtactcaaccaagtcattctgagaatagtgtatgcggcgaccgagttgctcttgcccggcgtcaatacgggataataccgcgccacatagcagaactttaaaagtgctcatcattggaaaacgttcttcggggcgaaaactctcaaggatcttaccgctgttgagatccagttcgatgtaacccactcgtgcacccaactgatcttcagcatcttttactttcaccagcgtttctgggtgagcaaaaacaggaaggcaaaatgccgcaaaaaagggaataagggcgacacggaaatgttgaatactcatactcttcctttttcaatattattgaagcatttatcagggttattgtctcatgagcggatacatatttgaatgtatttagaaaaataaacaaataggggttccgcgcacatttccccgaaaagtgccacctgacgtc

SEQ ID NO: 30 - DNA, 1977 bp, synthetic construct
  source 1..1977: mol_type = other DNA
atggcgccctttcctgaagaagtggacgtcttcaccgccccacactggcggatgaagcagctggtggggctctactgcgacaagctttctaaaaccaatttttccaacaacaacgatttccgtgctcttctgcagtctttgtatgctactttcaaggagttcaaaatgcatgagcagattgaaaatgaatacattattggtttgcttcaacaacgcagccagaccatttataatgtacattctgacaataaactctccgagatgcttagcctctttgaaaagggactgaagaatgttaagaatgaatatgaacagttaaattatgcaaaacaactgaaagagagattggaggcttttacaagagattttcttcctcacatgaaagaggaagaggaggtttttcagcccatgttaatggaatattttacctatgaagagcttaaggatattaaaaagaaagtgattgcacaacactgctctggcggcggcgtgagtaagggggaggaagataacatggcctcacttccagcgactcacgaacttcacatttttgggtccatcaatggcgtggatttcgatatggtagggcaagggactggcaaccctaacgacggttacgaagaactcaatctgaaatcaacgaaaggggatttgcaattttccccatggatactcgtcccccatataggctatggattccaccaatatctgccgtatccagacggaatgtctccgtttcaagccgcaatggtagacggtagcggttaccaggtccaccggacgatgcaattcgaagatggggcctccctgacagtaaattatagatatacctatgaagggagtcacataaagggagaagctcaggtcaaaggaacgggtttcccggctgacggaccggtgatgaccaattcactgaccgccgccgattggtgccgctctaaaaaaacttacccaaatgataagactatcatttcaacttttaaatggagttacactacggggaatggtaagaggtacaggtcaacagccaggacaacttacacatttgccaagccaatggcggcgaactatttgaaaaatcagccaatgtacgttttccgaaaaaccgaattgaaacattctaagaccgagcttaatttcaaggaatggcaaaaagcatttacggatgtgatggggatggatgagctttacaagggtaccggaagcggagagggcaggggaagtcttctaacatgcggggacgtggaggaaaatcccggccccatggtctccaaaggagaggaagacaatatggccattatcaaagagtttatgcgatttaaagtgcacatggagggaagcgtcaacgggcatgagtttgagattgagggggaaggagagggaagaccttatgaagggacccagactgccaaactgaaagtcaccaagggcggacccctgccatttgcttgggacattctgagcccacaattcatgtatgggtccaaagcctatgttaaacacccggcagacatacctgactacctcaagctctcctttcctgaggggtttaaatgggagagggtgatgaactttgaagatggaggcgtcgtgacagtaactcaggatagcagcctgcaagacggggagtttatttacaaggttaaattgcgcggaaccaactttcccagcgatggacccgtgatgcagaagaaaacaatgggctgggaagcatcatccgaaagaatgtatcccgaagatggcgcgttgaagggggaaatcaaacaaaggctcaagttgaaagatggagggcactatgacgctgaggtcaaaaccacgtacaaggctaaaaaaccggtacaactgcccggagcatataatgttaatattaagctggacatcaccagccacaatgaggattacacaatagtggaacagtatgaaagagccgagggaagacactcaactgggggcatggatgaactgtataaatgataa

SEQ ID NO: 31 - DNA, 56 bp, synthetic construct
  source 1..56: mol_type = other DNA
ttgtcacaatcctaacacattatcgggagcagtgtcttccataatgtataaagaac

SEQ ID NO: 32 - DNA, 93 bp, synthetic construct
  source 1..93: mol_type = other DNA
accacagtgtctgtatcggagacagtgatctccatatgttacactaagggtgtaagtaattatcgggaacagtgtttcccataattttcttca